European Patent Application EP 4 190 800 A1, published June 7, 2023. Title: Peptide for treating coronavirus disease COVID-19 and use thereof. Applicant: Daegu Gyeongbuk Institute of Science and Technology. The sequence listing filed with the application follows.

SEQUENCE LISTING (2 sequences)

SEQ ID NO: 1 - protein, 54 aa, Artificial Sequence
  PEP9 peptide
MKSQLADNVYNTNITKENVQNMNEEQAKTFLDKFNHEAEDLFYQSSGLGKGDFR

SEQ ID NO: 2 - DNA, 162 bp, Artificial Sequence
  PEP9 peptide
atgaaaagtcaacttgctgataatgtgtataacaccaatattactaaagagaatgtccaaaacatgaatgaggaacaggccaagacatttttggacaagtttaaccacgaagccgaagacctgttctatcaaagttcaggcctggggaagggcgacttcagg